European Patent Specification EP 3 898 698 B1, published April 1, 2026. Title: ANTIBODIES SPECIFIC TO MUC18. Applicant: Multitude Inc. Application Not Yet Assigned. The sequence listing filed with the application follows.

SEQUENCE LISTING (46 sequences)

SEQ ID NO: 1 - protein, 118 aa, Homo sapiens
QVQLQESGPGLVKPSETLSLTCTVSGYSITSGYYWNWIRQFPGNGLEWIGYINYGGTNNYNPSLKIRVTISRDTSKNQFSLKLSSVTAADTAVYYCARGNNDGGFAYWGQGTLVTVSS

SEQ ID NO: 2 - protein, 108 aa, Artificial Sequence
  Synthetic Polypeptide
DNQMTQSPSSLSASVGDRVTITCSASSSVSSTYLHWYQQKPGKSPKLLLYRASNLASGVPSRFSGSGSGTDYTLTISSLQPEDFATYYCHQWSGYPYTFGGGTKVEIK

SEQ ID NO: 3 - protein, 646 aa, Artificial Sequence
  Synthetic Polypeptide
MGLPRLVCAFLLAACCCCPRVAGVPGEAEQPAPELVEVEVGSTALLKCGLSQSQGNLSHVDWFSVHKEKRTLIFRVRQGQGQSEPGEYEQRLSLQDRGATLALTQVTPQDERIFLCQGKRPRSQEYRIQLRVYKAPEEPNIQVNPLGIPVNSKEPEEVATCVGRNGYPIPQVIWYKNGRPLKEEKNRVHIQSSQTVESSGLYTLQSILKAQLVKEDKDAQFYCELNYRLPSGNHMKESREVTVPVFYPTEKVWLEVEPVGMLKEGDRVEIRCLADGNPPPHFSISKQNPSTREAEEETTNDNGVLVLEPARKEHSGRYECQGLDLDTMISLLSEPQELLVNYVSDVRVSPAAPERQEGSSLTLTCEAESSQDLEFQWLREETGQVLERGPVLQLHDLKREAGGGYRCVASVPSIPGLNRTQLVNVAIFGPPWMAFKERKVWVKENMVLNLSCEASGHPRPTISWNVNGTASEQDQDPQRVLSTLNVLVTPELLETGVECTASNDLGKNTSILFLELVNLTTLTPDSNTTTGLSTSTASPHTRANSTSTERKLPEPESRGVVIVAVIVCILVLAVLGAVLYFLYKKGKLPCRRSGKQEITLPPSRKSELVVEVKSDKLPEEMGLLQGSSGDKRAPGDQGEKYIDLRH

SEQ ID NO: 4 - protein, 9 aa, Artificial Sequence
  Synthetic Polypeptide
GYSITSGYY

SEQ ID NO: 5 - protein, 7 aa, Artificial Sequence
  Synthetic Polypeptide
INYGGTN

SEQ ID NO: 6 - protein, 11 aa, Artificial Sequence
  Synthetic Polypeptide
ARGNNDGGFAY

SEQ ID NO: 7 - protein, 7 aa, Artificial Sequence
  Synthetic Polypeptide
SSVSSTY

SEQ ID NO: 8 - protein, 9 aa, Artificial Sequence
  Synthetic Polypeptide
HQWSGYPYT

SEQ ID NO: 9 - protein, 118 aa, Artificial Sequence
  Synthetic Polypeptide
DVQLQESGPGLVKPSQSLSLTCSVTGYSITSGYYWNWIRQFPGNKLEWLGYINYGGTNNYNPSLKIRGSITRDTSKNQFFLKLNSVTTEDTATYYCARGNNDGGFAYWGQGTLVTVSA

SEQ ID NO: 10 - protein, 108 aa, Artificial Sequence
  Synthetic Polypeptide
ENVLTQSPAIVAASLGQKVTMTCSASSSVSSTYLHWYQQKSGASPKPLLHRASNLASGVPARFSGSGSGTSYSLTISSVEAEDDATYYCHQWSGYPYTFGGGTKLEIK

SEQ ID NO: 11 - DNA, 33 bp, Artificial Sequence
  Synthetic Polynucleotide
gggaattcatgrasttskggytmarctkgrttt

SEQ ID NO: 12 - DNA, 34 bp, Artificial Sequence
  Synthetic Polynucleotide
gggaattcatgraatgsasctgggtywtyctctt

SEQ ID NO: 13 - DNA, 39 bp, Artificial Sequence
  Synthetic Polynucleotide
actagtcgacatggactccaggctcaatttagttttcct

SEQ ID NO: 14 - DNA, 36 bp, Artificial Sequence
  Synthetic Polynucleotide
actagtcgacatggctgtcytrgbgctgytcytctg

SEQ ID NO: 15 - DNA, 39 bp, Artificial Sequence
  Synthetic Polynucleotide
actagtcgacatggvttggstgtggamcttgcyattcct

SEQ ID NO: 16 - DNA, 36 bp, Artificial Sequence
  Synthetic Polynucleotide
actagtcgacatgaaatgcagctggrtyatsttctt

SEQ ID NO: 17 - DNA, 36 bp, Artificial Sequence
  Synthetic Polynucleotide
actagtcgacatggrcagrcttacwtyytcattcct

SEQ ID NO: 18 - DNA, 36 bp, Artificial Sequence
  Synthetic Polynucleotide
actagtcgacatgatggtgttaagtcttctgtacct

SEQ ID NO: 19 - DNA, 36 bp, Artificial Sequence
  Synthetic Polynucleotide
actagtcgacatgggatggagctrtatcatsytctt

SEQ ID NO: 20 - DNA, 33 bp, Artificial Sequence
  Synthetic Polynucleotide
actagtcgacatgaagwtgtggbtraactggrt

SEQ ID NO: 21 - DNA, 35 bp, Artificial Sequence
  Synthetic Polynucleotide
  misc_feature (25)..(25): n is inosine
actagtcgacatggratggasckknrtctttmtct

SEQ ID NO: 22 - DNA, 35 bp, Artificial Sequence
  Synthetic Polynucleotide
actagtcgacatgaacttygggytsagmttgrttt

SEQ ID NO: 23 - DNA, 35 bp, Artificial Sequence
  Synthetic Polynucleotide
actagtcgacatgtacttgggactgagctgtgtat

SEQ ID NO: 24 - DNA, 33 bp, Artificial Sequence
  Synthetic Polynucleotide
actagtcgacatgagagtgctgattcttttgtg

SEQ ID NO: 25 - DNA, 38 bp, Artificial Sequence
  Synthetic Polynucleotide
actagtcgacatggattttgggctgattttttttattg

SEQ ID NO: 26 - DNA, 32 bp, Artificial Sequence
  Synthetic Polynucleotide
cccaagcttacgagggggaagacatttgggaa

SEQ ID NO: 27 - DNA, 35 bp, Artificial Sequence
  Synthetic Polynucleotide
  misc_feature (30)..(30): n is inosine
cccaagcttccagggrccarkggataracngrtgg

SEQ ID NO: 28 - DNA, 32 bp, Artificial Sequence
  Synthetic Polynucleotide
gggaattcatgragwcacakwcycaggtcttt

SEQ ID NO: 29 - DNA, 33 bp, Artificial Sequence
  Synthetic Polynucleotide
gggaattcatggagacagacacactcctgctat

SEQ ID NO: 30 - DNA, 39 bp, Artificial Sequence
  Synthetic Polynucleotide
actagtcgacatggagwcagacacactsctgytatgggt

SEQ ID NO: 31 - DNA, 42 bp, Artificial Sequence
  Synthetic Polynucleotide
  misc_feature (37)..(37): n is inosine
actagtcgacatgaggrcccctgctcagwttyttggnwtctt

SEQ ID NO: 32 - DNA, 41 bp, Artificial Sequence
  Synthetic Polynucleotide
actagtcgacatgggcwtcaagatgragtcacakwyycwgg

SEQ ID NO: 33 - DNA, 39 bp, Artificial Sequence
  Synthetic Polynucleotide
actagtcgacatgagtgtgcycactcaggtcctggsgtt

SEQ ID NO: 34 - DNA, 41 bp, Artificial Sequence
  Synthetic Polynucleotide
actagtcgacatgtggggaycgktttyammcttttcaattg

SEQ ID NO: 35 - DNA, 38 bp, Artificial Sequence
  Synthetic Polynucleotide
actagtcgacatggaagccccagctcagcttctcttcc

SEQ ID NO: 36 - DNA, 36 bp, Artificial Sequence
  Synthetic Polynucleotide
  misc_feature (16)..(16): n is inosine
  misc_feature (22)..(22): n is inosine
  misc_feature (28)..(28): n is inosine
actagtcgacatgagnmmktcnmttcanttcytggg

SEQ ID NO: 37 - DNA, 36 bp, Artificial Sequence
  Synthetic Polynucleotide
  misc_feature (22)..(22): n is inosine
  misc_feature (34)..(34): n is inosine
actagtcgacatgakgthcycngctcagytyctnrg

SEQ ID NO: 38 - DNA, 35 bp, Artificial Sequence
  Synthetic Polynucleotide
actagtcgacatggtrtccwcasctcagttccttg

SEQ ID NO: 39 - DNA, 37 bp, Artificial Sequence
  Synthetic Polynucleotide
actagtcgacatgtatatatgtttgttgtctatttct

SEQ ID NO: 40 - DNA, 39 bp, Artificial Sequence
  Synthetic Polynucleotide
actagtcgacatgaagttgcctgttaggctgttggtgct

SEQ ID NO: 41 - DNA, 39 bp, Artificial Sequence
  Synthetic Polynucleotide
actagtcgacatggatttwcargtgcagattwtcagctt

SEQ ID NO: 42 - DNA, 37 bp, Artificial Sequence
  Synthetic Polynucleotide
actagtcgacatggtyctyatvtccttgctgttctgg

SEQ ID NO: 43 - DNA, 37 bp, Artificial Sequence
  Synthetic Polynucleotide
actagtcgacatggtyctyatvttrctgctgctatgg

SEQ ID NO: 44 - DNA, 30 bp, Artificial Sequence
  Synthetic Polynucleotide
cccaagcttactggatggtgggaagatgga

SEQ ID NO: 45 - DNA, 33 bp, Artificial Sequence
  Synthetic Polynucleotide
gggaattcatggcctggaytycwctywtmytct

SEQ ID NO: 46 - DNA, 32 bp, Artificial Sequence
  Synthetic Polynucleotide
  misc_feature (24)..(24): n is inosine
cccaagcttagctcytcwgwgganggyggraa